European Patent Application EP 4 119 571 A1, published January 18, 2023. Title: A novel bispecific protein and use thereof. Applicant: SL METAGEN. The sequence listing filed with the application follows.

SEQUENCE LISTING (69 sequences)

SEQ ID NO: 1 - protein, 31 aa, Artificial Sequence
  human GLP-1 mutant (A2G)
HGEGTFTSDVSSYLEGQAAKEFIAWLVKGRG

SEQ ID NO: 2 - protein, 31 aa, Artificial Sequence
  human GLP-1 wild type
HAEGTFTSDVSSYLEGQAAKEFIAWLVKGRG

SEQ ID NO: 3 - protein, 39 aa, Artificial Sequence
  Exendin 3
HSDGTFTSDLSKQMEEEAVRLFIEWLKNGGPSSGAPPPS

SEQ ID NO: 4 - protein, 39 aa, Artificial Sequence
  Exendin 4
HGEGTFTSDLSKQMEEEAVRLFIEWLKNGGPSSGAPPPS

SEQ ID NO: 5 - protein, 39 aa, Artificial Sequence
  GLP-1/Exendin 4 hybrid
HGEGTFTSDVSSYLEGQAAKEFIAWLVKGGPSSGAPPPS

SEQ ID NO: 6 - protein, 44 aa, Artificial Sequence
  Lixisenatide
HGEGTFTSDLSKQMEEEAVRLFIEWLKNGGPSSGAPPSKKKKKK

SEQ ID NO: 7 - protein, 905 aa, Artificial Sequence
  Exendin 4-XTEN
HGEGTFTSDLSKQMEEEAVRLFIEWLKNGGPSSGAPPPSGGSPAGSPTSTEEGTSESATPESGPGTSTEPSEGSAPGSPAGSPTSTEEGTSTEPSEGSAPGTSTEPSEGSAPGTSESATPESGPGSEPATSGSETPGSEPATSGSETPGSPAGSPTSTEEGTSESATPESGPGTSTEPSEGSAPGTSTEPSEGSAPGSPAGSPTSTEEGTSTEPSEGSAPGTSTEPSEGSAPGTSESATPESGPGTSTEPSEGSAPGTSESATPESGPGSEPATSGSETPGTSTEPSEGSAPGTSTEPSEGSAPGTSESATPESGPGTSESATPESGPGSPAGSPTSTEEGTSESATPESGPGSEPATSGSETPGTSESATPESGPGTSTEPSEGSAPGTSTEPSEGSAPGTSTEPSEGSAPGTSTEPSEGSAPGTSTEPSEGSAPGTSTEPSEGSAPGSPAGSPTSTEEGTSTEPSEGSAPGTSESATPESGPGSEPATSGSETPGTSESATPESGPGSEPATSGSETPGTSESATPESGPGTSTEPSEGSAPGTSESATPESGPGSPAGSPTSTEEGSPAGSPTSTEEGSPAGSPTSTEEGTSESATPESGPGTSTEPSEGSAPGTSESATPESGPGSEPATSGSETPGTSESATPESGPGSEPATSGSETPGTSESATPESGPGTSTEPSEGSAPGSPAGSPTSTEEGTSESATPESGPGSEPATSGSETPGTSESATPESGPGSPAGSPTSTEEGSPAGSPTSTEEGTSTEPSEGSAPGTSESATPESGPGTSESATPESGPGTSESATPESGPGSEPATSGSETPGSEPATSGSETPGSPAGSPTSTEEGTSTEPSEGSAPGTSTEPSEGSAPGSEPATSGSETPGTSESATPESGPGTSTEPSEGSAPG

SEQ ID NO: 8 - protein, 645 aa, Artificial Sequence
  Albiglutide
HGEGTFTSDVSSYLEGQAAKEFIAWLVKGRHGEGTFTSDVSSYLEGQAAKEFIAWLVKGRDAHKSEVAHRFKDLGEENFKALVLIAFAQYLQQCPFEDHVKLVNEVTEFAKTCVADESAENCDKSLHTLFGDKLCTVATLRETYGEMADCCAKQEPERNECFLQHKDDNPNLPRLVRPEVDVMCTAFHDNEETFLKKYLYEIARRHPYFYAPELLFFAKRYKAAFTECCQAADKAACLLPKLDELRDEGKASSAKQRLKCASLQKFGERAFKAWAVARLSQRFPKAEFAEVSKLVTDLTKVHTECCHGDLLECADDRADLAKYICENQDSISSKLKECCEKPLLEKSHCIAEVENDEMPADLPSLAADFVESKDVCKNYAEAKDVFLGMFLYEYARRHPDYSVVLLLRLAKTYETTLEKCCAAADPHECYAKVFDEFKPLVEEPQNLIKQNCELFEQLGEYKFQNALLVRYTKKVPQVSTPTLVEVSRNLGKVGSKCCKHPEAKRMPCAEDYLSVVLNQLCVLHEKTPVSDRVTKCCTESLVNRRPCFSALEVDETYVPKEFNAETFTFHADICTLSEKERQIKKQTALVELVKHKPKATKEQLKAVMDDFAAFVEKCCKADDKETCFAEEGKKLVAASQAALGL

SEQ ID NO: 9 - protein, 31 aa, Artificial Sequence
  Liraglutide
HAEGTFTSDVSSYLEGQAAKEFIAWLVRGRG

SEQ ID NO: 10 - protein, 30 aa, Artificial Sequence
  Taspoglutide
  MOD_RES (2): METHYLATION,
  MOD_RES (29): METHYLATION,
HXEGTFTSDVSSYLEGQAAKEFIAWLVKXR

SEQ ID NO: 11 - protein, 108 aa, Artificial Sequence
  GLP-1 tandem repeat
HGEGTFTSDVSSYLEGQAAKEFIAWLVKGGPSSGAPPPSGGGGSGGGGSGGGGSGGGGSGGGGSGGGGSHGEGTFTSDVSSYLEGQAAKEFIAWLVKGGPSSGAPPPS

SEQ ID NO: 12 - protein, 215 aa, Artificial Sequence
  hybrid Fc region
SHTQPLGVFLFPPKPKDTLMISRTPEVTCVVVDVSQEDPEVQFNWYVDGVEVHNAKTKPREEQFNSTYRVVSVLTVLHQDWLNGKEYKCKVSNKGLPSSIEKTISKAKGQPREPQVYTLPPSQEEMTKNQVSLTCLVKGFYPSDIAVEWESNGQPENNYKTTPPVLDSDGSFFLYSRLTVDKSRWQEGNVFSCSVMHEALHNHYTQKSLSLSLGK

SEQ ID NO: 13 - protein, 215 aa, Artificial Sequence
  hybrid Fc hole
SHTQPLGVFLFPPKPKDTLMISRTPEVTCVVVDVSQEDPEVQFNWYVDGVEVHNAKTKPREEQFNSTYRVVSVLTVLHQDWLNGKEYKCKVSNKGLPSSIEKTISKAKGQPREPQVCTLPPSQEEMTKNQVSLSCAVKGFYPSDIAVEWESNGQPENNYKTTPPVLDSDGSFFLVSRLTVDKSRWQEGNVFSCSVMHEALHNHYTQKSLSLSLGK

SEQ ID NO: 14 - protein, 215 aa, Artificial Sequence
  hybrid Fc knob
SHTQPLGVFLFPPKPKDTLMISRTPEVTCVVVDVSQEDPEVQFNWYVDGVEVHNAKTKPREEQFNSTYRVVSVLTVLHQDWLNGKEYKCKVSNKGLPSSIEKTISKAKGQPREPQVYTLPPCQEEMTKNQVSLWCLVKGFYPSDIAVEWESNGQPENNYKTTPPVLDSDGSFFLYSRLTVDKSRWQEGNVFSCSVMHEALHNHYTQKSLSLSLGK

SEQ ID NO: 15 - protein, 215 aa, Artificial Sequence
  hybrid Fc knob
SHTQPLGVFLFPPKPKDQLMISRTPEVTCVVVDVSQEDPEVQFNWYVDGVEVHNAKTKPREEQFNSTYRVVSVLTVLHQDWLNGKEYKCKVSNKGLPSSIEKTISKAKGQPREPQVYTLPPCQEEMTKNQVSLWCLVKGFYPSDIAVEWESNGQPENNYKTTPPVLDSDGSFFLYSRLTVDKSRWQEGNVFSCSVLHEALHNHYTQKSLSLSLGK

SEQ ID NO: 16 - protein, 215 aa, Artificial Sequence
  hybrid Fc hole
SHTQPLGVFLFPPKPKDQLMISRTPEVTCVVVDVSQEDPEVQFNWYVDGVEVHNAKTKPREEQFNSTYRVVSVLTVLHQDWLNGKEYKCKVSNKGLPSSIEKTISKAKGQPREPQVCTLPPSQEEMTKNQVSLSCAVKGFYPSDIAVEWESNGQPENNYKTTPPVLDSDGSFFLVSRLTVDKSRWQEGNVFSCSVLHEALHNHYTQKSLSLSLGK

SEQ ID NO: 17 - protein, 33 aa, Artificial Sequence
  human GLP-2 mutant (A2G)
HGDGSFSDEMNTILDNLAARDFINWLIQTKITD

SEQ ID NO: 18 - protein, 33 aa, Artificial Sequence
  human GLP-2 wild type
HADGSFSDEMNTILDNLAARDFINWLIQTKITD

SEQ ID NO: 19 - protein, 33 aa, Artificial Sequence
  human GLP-2 mutant (A2G, N16G, L17Q)
HGDGSFSDEMNTILDGQAARDFINWLIQTKITD

SEQ ID NO: 20 - protein, 33 aa, Artificial Sequence
  human GLP-2 mutant (A2G, L17Q)
HGDGSFSDEMNTILDNQAARDFINWLIQTKITD

SEQ ID NO: 21 - protein, 39 aa, Artificial Sequence
  Glepaglutide
HGEGTFSSELATILDALAARDFIAWLIATKITDKKKKKK

SEQ ID NO: 22 - protein, 42 aa, Artificial Sequence
  GLP-2 analogue 10
  MOD_RES (11): linked with a lipidated cross-linker via thiol groups of 11th and 18th amino acids, cystein
  MOD_RES (18): linked with a lipidated cross-linker via thiol groups of 11th and 18th amino acids, cystein
HGDGSFSDEMCTILDNLCARDFINWLIQTKITDPSSGAPPPS

SEQ ID NO: 23 - protein, 286 aa, Artificial Sequence
  first fusion protein of bispecific fusion protein containing GLP-1 analogue
HGEGTFTSDVSSYLEGQAAKEFIAWLVKGRGAKATTAPATTRNTGRGGEEKKKEKEKEEQEERETKTPECPSHTQPLGVFLFPPKPKDTLMISRTPEVTCVVVDVSQEDPEVQFNWYVDGVEVHNAKTKPREEQFNSTYRVVSVLTVLHQDWLNGKEYKCKVSNKGLPSSIEKTISKAKGQPREPQVYTLPPSQEEMTKNQVSLTCLVKGFYPSDIAVEWESNGQPENNYKTTPPVLDSDGSFFLYSRLTVDKSRWQEGNVFSCSVMHEALHNHYTQKSLSLSLGK

SEQ ID NO: 24 - protein, 301 aa, Artificial Sequence
  first fusion protein of bispecific fusion protein containing GLP-1 analogue
HGEGTFTSDVSSYLEGQAAKEFIAWLVKGRGGGGGSGGGGSGGGGSAKNTTAPATTRNTTRGGEEKKKEKEKEEQEERTHTCPPCPSHTQPLGVFLFPPKPKDTLMISRTPEVTCVVVDVSQEDPEVQFNWYVDGVEVHNAKTKPREEQFNSTYRVVSVLTVLHQDWLNGKEYKCKVSNKGLPSSIEKTISKAKGQPREPQVYTLPPCQEEMTKNQVSLWCLVKGFYPSDIAVEWESNGQPENNYKTTPPVLDSDGSFFLYSRLTVDKSRWQEGNVFSCSVMHEALHNHYTQKSLSLSLGK

SEQ ID NO: 25 - protein, 279 aa, Artificial Sequence
  first fusion protein of bispecific fusion protein containing GLP-1 analogue
HGEGTFTSDVSSYLEGQAAKEFIAWLVKGRGGGGGSGGGGSGGGGSEKEKEEQEERTHTCPPCPSHTQPLGVFLFPPKPKDTLMISRTPEVTCVVVDVSQEDPEVQFNWYVDGVEVHNAKTKPREEQFNSTYRVVSVLTVLHQDWLNGKEYKCKVSNKGLPSSIEKTISKAKGQPREPQVCTLPPSQEEMTKNQVSLSCAVKGFYPSDIAVEWESNGQPENNYKTTPPVLDSDGSFFLVSRLTVDKSRWQEGNVFSCSVMHEALHNHYTQKSLSLSLGK

SEQ ID NO: 26 - protein, 309 aa, Artificial Sequence
  first fusion protein of bispecific fusion protein containing GLP-1 analogue
HGEGTFTSDLSKQMEEEAVRLFIEWLKNGGPSSGAPPPSGGGGSGGGGSGGGGSAKNTTAPATTRNTTRGGEEKKKEKEKEEQEERTHTCPPCPSHTQPLGVFLFPPKPKDTLMISRTPEVTCVVVDVSQEDPEVQFNWYVDGVEVHNAKTKPREEQFNSTYRVVSVLTVLHQDWLNGKEYKCKVSNKGLPSSIEKTISKAKGQPREPQVYTLPPCQEEMTKNQVSLWCLVKGFYPSDIAVEWESNGQPENNYKTTPPVLDSDGSFFLYSRLTVDKSRWQEGNVFSCSVMHEALHNHYTQKSLSLSLGK

SEQ ID NO: 27 - protein, 310 aa, Artificial Sequence
  first fusion protein of bispecific fusion protein containing GLP-1 analogue
HGEGTFTSDVSSYLEGQAAKEFIAWLVKGGPSSGAPPPSGGGGGSGGGGSGGGGSAKNTTAPATTRNTTRGGEEKKKEKEKEEQEERTHTCPPCPSHTQPLGVFLFPPKPKDQLMISRTPEVTCVVVDVSQEDPEVQFNWYVDGVEVHNAKTKPREEQFNSTYRVVSVLTVLHQDWLNGKEYKCKVSNKGLPSSIEKTISKAKGQPREPQVYTLPPCQEEMTKNQVSLWCLVKGFYPSDIAVEWESNGQPENNYKTTPPVLDSDGSFFLYSRLTVDKSRWQEGNVFSCSVLHEALHNHYTQKSLSLSLGK

SEQ ID NO: 28 - protein, 287 aa, Artificial Sequence
  first fusion protein of bispecific fusion protein containing GLP-1 analogue
HGEGTFTSDVSSYLEGQAAKEFIAWLVKGGPSSGAPPPSGGGGSGGGGSGGGGSEKEKEEQEERTHTCPPCPSHTQPLGVFLFPPKPKDQLMISRTPEVTCVVVDVSQEDPEVQFNWYVDGVEVHNAKTKPREEQFNSTYRVVSVLTVLHQDWLNGKEYKCKVSNKGLPSSIEKTISKAKGQPREPQVYTLPPCQEEMTKNQVSLWCLVKGFYPSDIAVEWESNGQPENNYKTTPPVLDSDGSFFLYSRLTVDKSRWQEGNVFSCSVLHEALHNHYTQKSLSLSLGK

SEQ ID NO: 29 - protein, 309 aa, Artificial Sequence
  first fusion protein of bispecific fusion protein containing GLP-1 analogue
HGEGTFTSDVSSYLEGQAAKEFIAWLVKGGPSSGAPPPSGGGGSGGGGSGGGGSAKNTTAPATTRNTTRGGEEKKKEKEKEEQEERTHTCPPCPSHTQPLGVFLFPPKPKDQLMISRTPEVTCVVVDVSQEDPEVQFNWYVDGVEVHNAKTKPREEQFNSTYRVVSVLTVLHQDWLNGKEYKCKVSNKGLPSSIEKTISKAKGQPREPQVYTLPPCQEEMTKNQVSLWCLVKGFYPSDIAVEWESNGQPENNYKTTPPVLDSDGSFFLYSRLTVDKSRWQEGNVFSCSVLHEALHNHYTQKSLSLSLGK

SEQ ID NO: 30 - protein, 353 aa, Artificial Sequence
  first fusion protein of bispecific fusion protein containing GLP-1 analogue
HGEGTFTSDVSSYLEGQAAKEFIAWLVKGGPSSGAPPPSGGGGSGGGGSGGGGSGGGGSGGGGSGGGGSHGEGTFTSDVSSYLEGQAAKEFIAWLVKGGPSSGAPPPSGGGGSGGGGSGGGGSEPKSSDKTHTCPPCPSHTQPLGVFLFPPKPKDQLMISRTPEVTCVVVDVSQEDPEVQFNWYVDGVEVHNAKTKPREEQFNSTYRVVSVLTVLHQDWLNGKEYKCKVSNKGLPSSIEKTISKAKGQPREPQVYTLPPCQEEMTKNQVSLWCLVKGFYPSDIAVEWESNGQPENNYKTTPPVLDSDGSFFLYSRLTVDKSRWQEGNVFSCSVLHEALHNHYTQKSLSLSLGK

SEQ ID NO: 31 - protein, 288 aa, Artificial Sequence
  second fusion protein of bispecific fusion protein containing GLP-2 analogue
HGDGSFSDEMNTILDNLAARDFINWLIQTKITDAKATTAPATTRNTGRGGEEKKKEKEKEEQEERETKTPECPSHTQPLGVFLFPPKPKDTLMISRTPEVTCVVVDVSQEDPEVQFNWYVDGVEVHNAKTKPREEQFNSTYRVVSVLTVLHQDWLNGKEYKCKVSNKGLPSSIEKTISKAKGQPREPQVYTLPPSQEEMTKNQVSLTCLVKGFYPSDIAVEWESNGQPENNYKTTPPVLDSDGSFFLYSRLTVDKSRWQEGNVFSCSVMHEALHNHYTQKSLSLSLGK

SEQ ID NO: 32 - protein, 281 aa, Artificial Sequence
  second fusion protein of bispecific fusion protein containing GLP-2 analogue
HGDGSFSDEMNTILDNLAARDFINWLIQTKITDGGGGSGGGGSGGGGSEKEKEEQEERTHTCPPCPSHTQPLGVFLFPPKPKDTLMISRTPEVTCVVVDVSQEDPEVQFNWYVDGVEVHNAKTKPREEQFNSTYRVVSVLTVLHQDWLNGKEYKCKVSNKGLPSSIEKTISKAKGQPREPQVCTLPPSQEEMTKNQVSLSCAVKGFYPSDIAVEWESNGQPENNYKTTPPVLDSDGSFFLVSRLTVDKSRWQEGNVFSCSVMHEALHNHYTQKSLSLSLGK

SEQ ID NO: 33 - protein, 303 aa, Artificial Sequence
  second fusion protein of bispecific fusion protein containing GLP-2 analogue
HGDGSFSDEMNTILDNLAARDFINWLIQTKITDGGGGSGGGGSGGGGSAKNTTAPATTRNTTRGGEEKKKEKEKEEQEERTHTCPPCPSHTQPLGVFLFPPKPKDTLMISRTPEVTCVVVDVSQEDPEVQFNWYVDGVEVHNAKTKPREEQFNSTYRVVSVLTVLHQDWLNGKEYKCKVSNKGLPSSIEKTISKAKGQPREPQVYTLPPCQEEMTKNQVSLWCLVKGFYPSDIAVEWESNGQPENNYKTTPPVLDSDGSFFLYSRLTVDKSRWQEGNVFSCSVMHEALHNHYTQKSLSLSLGK

SEQ ID NO: 34 - protein, 281 aa, Artificial Sequence
  second fusion protein of bispecific fusion protein containing GLP-2 analogue
HGDGSFSDEMNTILDNLAARDFINWLIQTKITDGGGGSGGGGSGGGGSEKEKEEQEERTHTCPPCPSHTQPLGVFLFPPKPKDQLMISRTPEVTCVVVDVSQEDPEVQFNWYVDGVEVHNAKTKPREEQFNSTYRVVSVLTVLHQDWLNGKEYKCKVSNKGLPSSIEKTISKAKGQPREPQVCTLPPSQEEMTKNQVSLSCAVKGFYPSDIAVEWESNGQPENNYKTTPPVLDSDGSFFLVSRLTVDKSRWQEGNVFSCSVLHEALHNHYTQKSLSLSLGK

SEQ ID NO: 35 - protein, 304 aa, Artificial Sequence
  second fusion protein of bispecific fusion protein containing GLP-2 analogue
HGDGSFSDEMNTILDNLAARDFINWLIQTKITDGGGGGSGGGGSGGGGSAKNTTAPATTRNTTRGGEEKKKEKEKEEQEERTHTCPPCPSHTQPLGVFLFPPKPKDQLMISRTPEVTCVVVDVSQEDPEVQFNWYVDGVEVHNAKTKPREEQFNSTYRVVSVLTVLHQDWLNGKEYKCKVSNKGLPSSIEKTISKAKGQPREPQVCTLPPSQEEMTKNQVSLSCAVKGFYPSDIAVEWESNGQPENNYKTTPPVLDSDGSFFLVSRLTVDKSRWQEGNVFSCSVLHEALHNHYTQKSLSLSLGK

SEQ ID NO: 36 - protein, 278 aa, Artificial Sequence
  second fusion protein of bispecific fusion protein containing GLP-2 analogue
HGDGSFSDEMNTILDGQAARDFINWLIQTKITDGGGGSGGGGSGGGGSEPKSSDKTHTCPPCPSHTQPLGVFLFPPKPKDQLMISRTPEVTCVVVDVSQEDPEVQFNWYVDGVEVHNAKTKPREEQFNSTYRVVSVLTVLHQDWLNGKEYKCKVSNKGLPSSIEKTISKAKGQPREPQVCTLPPSQEEMTKNQVSLSCAVKGFYPSDIAVEWESNGQPENNYKTTPPVLDSDGSFFLVSRLTVDKSRWQEGNVFSCSVLHEALHNHYTQKSLSLSLGK

SEQ ID NO: 37 - protein, 15 aa, Artificial Sequence
  linker peptide
EPKSSDKTHTCPPCP

SEQ ID NO: 38 - protein, 15 aa, Artificial Sequence
  linker peptide
EPKSCDKTHTCPPCP

SEQ ID NO: 39 - protein, 30 aa, Artificial Sequence
  linker peptide
GGGGSGGGGSGGGGSEPKSSDKTHTCPPCP

SEQ ID NO: 40 - protein, 30 aa, Artificial Sequence
  linker peptide
GGGGSGGGGSGGGGSEPKSCDKTHTCPPCP

SEQ ID NO: 41 - protein, 40 aa, Artificial Sequence
  linker peptide
AKATTAPATTRNTGRGGEEKKKEKEKEEQEERETKTPECP

SEQ ID NO: 42 - protein, 33 aa, Artificial Sequence
  linker peptide
GGGGSGGGGSGGGGSEKEKEEQEERTHTCPPCP

SEQ ID NO: 43 - protein, 55 aa, Artificial Sequence
  linker peptide
GGGGSGGGGSGGGGSAKNTTAPATTRNTTRGGEEKKKEKEKEEQEERTHTCPPCP

SEQ ID NO: 44 - protein, 20 aa, Artificial Sequence
  linker peptide
AAGSGGGGGSGGGGSGGGGS

SEQ ID NO: 45 - protein, 15 aa, Artificial Sequence
  linker peptide
GGGGSGGGGSGGGGS

SEQ ID NO: 46 - protein, 5 aa, Artificial Sequence
  linker peptide
GGSGG

SEQ ID NO: 47 - protein, 9 aa, Artificial Sequence
  linker peptide
GGSGGSGGS

SEQ ID NO: 48 - protein, 6 aa, Artificial Sequence
  linker peptide
GGGSGG

SEQ ID NO: 49 - protein, 5 aa, Artificial Sequence
  linker peptide unit sequence
GGGGS

SEQ ID NO: 50 - protein, 6 aa, Artificial Sequence
  linker peptide unit sequence
GSSGGS

SEQ ID NO: 51 - protein, 18 aa, Artificial Sequence
  linker peptide
KESGSVSSEQLAQFRSLD

SEQ ID NO: 52 - protein, 14 aa, Artificial Sequence
  linker peptide
EGKSSGSGSESKST

SEQ ID NO: 53 - protein, 12 aa, Artificial Sequence
  linker peptide
GSAGSAAGSGEF

SEQ ID NO: 54 - protein, 5 aa, Artificial Sequence
  linker peptide unit sequence
EAAAK

SEQ ID NO: 55 - protein, 12 aa, Artificial Sequence
  linker peptide
CRRRRRREAEAC

SEQ ID NO: 56 - protein, 46 aa, Artificial Sequence
  linker peptide
AEAAAKEAAAKEAAAKEAAAKALEAEAAAKEAAAKEAAAKEAAAKA

SEQ ID NO: 57 - protein, 8 aa, Artificial Sequence
  linker peptide
GGGGGGGG

SEQ ID NO: 58 - protein, 6 aa, Artificial Sequence
  linker peptide
GGGGGG

SEQ ID NO: 59 - protein, 13 aa, Artificial Sequence
  linker peptide
AEAAAKEAAAAKA

SEQ ID NO: 60 - protein, 5 aa, Artificial Sequence
  linker peptide
PAPAP

SEQ ID NO: 61 - protein, 17 aa, Artificial Sequence
  linker peptide
VSQTSKLTRAETVFPDV

SEQ ID NO: 62 - protein, 6 aa, Artificial Sequence
  linker peptide
PLGLWA

SEQ ID NO: 63 - protein, 10 aa, Artificial Sequence
  linker peptide
TRHRQPRGWE

SEQ ID NO: 64 - protein, 10 aa, Artificial Sequence
  linker peptide
AGNRVRRSVG

SEQ ID NO: 65 - protein, 8 aa, Artificial Sequence
  linker peptide
RRRRRRRR

SEQ ID NO: 66 - protein, 4 aa, Artificial Sequence
  linker peptide
GFLG

SEQ ID NO: 67 - protein, 31 aa, Artificial Sequence
  linker peptide
GSSGGSGSSGGSGGGDEADGSRGSQKAGVDE

SEQ ID NO: 68 - protein, 15 aa, Artificial Sequence
  linker peptide
GSTSGSGKPGSGEGS

SEQ ID NO: 69 - protein, 103 aa, Artificial Sequence
  IgG1 CH3 domain
EPQVYTLPPSRDELTKNQVSLTCLVKGFYPSDIAVEWESNGQPENNYKTTPPVLDSDGSFFLYSKLTVDKSRWQQGNVFSCSVMHEALHNHYTQKSLSLSPGK